European Patent Specification EP 3 658 118 B1, published March 19, 2025. Title: METHODS AND COMPOSITIONS FOR  TREATING RESPIRATORY DISEASE. Applicant: Novavax, Inc. The sequence listing filed with the application follows.

SEQUENCE LISTING (20 sequences)

SEQ ID NO: 1 - DNA, 1725 bp, Respiratory syncytial virus
atggagttgctaatcctcaaagcaaatgcaattaccacaatcctcactgcagtcacattttgttttgcttctggtcaaaacatcactgaagaattttatcaatcaacatgcagtgcagttagcaaaggctatcttagtgctctgagaactggttggtataccagtgttataactatagaattaagtaatatcaaggaaaataagtgtaatggaacagatgctaaggtaaaattgataaaacaagaattagataaatataaaaatgctgtaacagaattgcagttgctcatgcaaagcacaccaccaacaaacaatcgagccagaagagaactaccaaggtttatgaattatacactcaacaatgccaaaaaaaccaatgtaacattaagcaagaaaaggaaaagaagatttcttggttttttgttaggtgttggatctgcaatcgccagtggcgttgctgtatctaaggtcctgcacctagaaggggaagtgaacaagatcaaaagtgctctactatccacaaacaaggctgtagtcagcttatcaaatggagttagtgtcttaaccagcaaagtgttagacctcaaaaactatatagataaacaattgttacctattgtgaacaagcaaagctgcagcatatcaaatatagaaactgtgatagagttccaacaaaagaacaacagactactagagattaccagggaatttagtgttaatgcaggtgtaactacacctgtaagcacttacatgttaactaatagtgaattattgtcattaatcaatgatatgcctataacaaatgatcagaaaaagttaatgtccaacaatgttcaaatagttagacagcaaagttactctatcatgtccataataaaagaggaagtcttagcatatgtagtacaattaccactatatggtgttatagatacaccctgttggaaactacacacatcccctctatgtacaaccaacacaaaagaagggtccaacatctgtttaacaagaactgacagaggatggtactgtgacaatgcaggatcagtatctttcttcccacaagctgaaacatgtaaagttcaatcaaatcgagtattttgtgacacaatgaacagtttaacattaccaagtgaaataaatctctgcaatgttgacatattcaaccccaaatatgattgtaaaattatgacttcaaaaacagatgtaagcagctccgttatcacatctctaggagccattgtgtcatgctatggcaaaactaaatgtacagcatccaataaaaatcgtggaatcataaagacattttctaacgggtgcgattatgtatcaaataaagggatggacactgtgtctgtaggtaacacattatattatgtaaataagcaagaaggtaaaagtctctatgtaaaaggtgaaccaataataaatttctatgacccattagtattcccctctgatgaatttgatgcatcaatatctcaagtcaacgagaagattaaccagagcctagcatttattcgtaaatccgatgaattattacataatgtaaatgctggtaaatccaccacaaatatcatgataactactataattatagtgattatagtaatattgttatcattaattgctgttggactgctcttatactgtaaggccagaagcacaccagtcacactaagcaaagatcaactgagtggtataaataatattgcatttagtaactaa

SEQ ID NO: 2 - protein, 574 aa, Respiratory syncytial virus
MELLILKANAITTILTAVTFCFASGQNITEEFYQSTCSAVSKGYLSALRTGWYTSVITIELSNIKENKCNGTDAKVKLIKQELDKYKNAVTELQLLMQSTPPTNNRARRELPRFMNYTLNNAKKTNVTLSKKRKRRFLGFLLGVGSAIASGVAVSKVLHLEGEVNKIKSALLSTNKAVVSLSNGVSVLTSKVLDLKNYIDKQLLPIVNKQSCSISNIETVIEFQQKNNRLLEITREFSVNAGVTTPVSTYMLTNSELLSLINDMPITNDQKKLMSNNVQIVRQQSYSIMSIIKEEVLAYVVQLPLYGVIDTPCWKLHTSPLCTTNTKEGSNICLTRTDRGWYCDNAGSVSFFPQAETCKVQSNRVFCDTMNSLTLPSEINLCNVDIFNPKYDCKIMTSKTDVSSSVITSLGAIVSCYGKTKCTASNKNRGIIKTFSNGCDYVSNKGMDTVSVGNTLYYVNKQEGKSLYVKGEPIINFYDPLVFPSDEFDASISQVNEKINQSLAFIRKSDELLHNVNAGKSTTNIMITTIIIVIIVILLSLIAVGLLLYCKARSTPVTLSKDQLSGINNIAFSN

SEQ ID NO: 3 - protein, 573 aa, Artificial Sequence
  Deletion of 137 (delta 1)
MELLILKANAITTILTAVTFCFASGQNITEEFYQSTCSAVSKGYLSALRTGWYTSVITIELSNIKENKCNGTDAKVKLIKQELDKYKNAVTELQLLMQSTPATNNRARRELPRFMNYTLNNAKKTNVTLSKKQKQQLGFLLGVGSAIASGVAVSKVLHLEGEVNKIKSALLSTNKAVVSLSNGVSVLTSKVLDLKNYIDKQLLPIVNKQSCSISNIETVIEFQQKNNRLLEITREFSVNAGVTTPVSTYMLTNSELLSLINDMPITNDQKKLMSNNVQIVRQQSYSIMSIIKEEVLAYVVQLPLYGVIDTPCWKLHTSPLCTTNTKEGSNICLTRTDRGWYCDNAGSVSFFPQAETCKVQSNRVFCDTMNSLTLPSEVNLCNVDIFNPKYDCKIMTSKTDVSSSVITSLGAIVSCYGKTKCTASNKNRGIIKTFSNGCDYVSNKGVDTVSVGNTLYYVNKQEGKSLYVKGEPIINFYDPLVFPSDEFDASISQVNEKINQSLAFIRKSDELLHNVNAGKSTTNIMITTIIIVIIVILLSLIAVGLLLYCKARSTPVTLSKDQLSGINNIAFSN

SEQ ID NO: 4 - protein, 572 aa, Artificial Sequence
  Deletion of 137-138 (delta 2)
MELLILKANAITTILTAVTFCFASGQNITEEFYQSTCSAVSKGYLSALRTGWYTSVITIELSNIKENKCNGTDAKVKLIKQELDKYKNAVTELQLLMQSTPATNNRARRELPRFMNYTLNNAKKTNVTLSKKQKQQGFLLGVGSAIASGVAVSKVLHLEGEVNKIKSALLSTNKAVVSLSNGVSVLTSKVLDLKNYIDKQLLPIVNKQSCSISNIETVIEFQQKNNRLLEITREFSVNAGVTTPVSTYMLTNSELLSLINDMPITNDQKKLMSNNVQIVRQQSYSIMSIIKEEVLAYVVQLPLYGVIDTPCWKLHTSPLCTTNTKEGSNICLTRTDRGWYCDNAGSVSFFPQAETCKVQSNRVFCDTMNSLTLPSEVNLCNVDIFNPKYDCKIMTSKTDVSSSVITSLGAIVSCYGKTKCTASNKNRGIIKTFSNGCDYVSNKGVDTVSVGNTLYYVNKQEGKSLYVKGEPIINFYDPLVFPSDEFDASISQVNEKINQSLAFIRKSDELLHNVNAGKSTTNIMITTIIIVIIVILLSLIAVGLLLYCKARSTPVTLSKDQLSGINNIAFSN

SEQ ID NO: 5 - protein, 571 aa, Artificial Sequence
  Deletion of 137-139 (delta 3)
MELLILKANAITTILTAVTFCFASGQNITEEFYQSTCSAVSKGYLSALRTGWYTSVITIELSNIKENKCNGTDAKVKLIKQELDKYKNAVTELQLLMQSTPATNNRARRELPRFMNYTLNNAKKTNVTLSKKQKQQFLLGVGSAIASGVAVSKVLHLEGEVNKIKSALLSTNKAVVSLSNGVSVLTSKVLDLKNYIDKQLLPIVNKQSCSISNIETVIEFQQKNNRLLEITREFSVNAGVTTPVSTYMLTNSELLSLINDMPITNDQKKLMSNNVQIVRQQSYSIMSIIKEEVLAYVVQLPLYGVIDTPCWKLHTSPLCTTNTKEGSNICLTRTDRGWYCDNAGSVSFFPQAETCKVQSNRVFCDTMNSLTLPSEVNLCNVDIFNPKYDCKIMTSKTDVSSSVITSLGAIVSCYGKTKCTASNKNRGIIKTFSNGCDYVSNKGVDTVSVGNTLYYVNKQEGKSLYVKGEPIINFYDPLVFPSDEFDASISQVNEKINQSLAFIRKSDELLHNVNAGKSTTNIMITTIIIVIIVILLSLIAVGLLLYCKARSTPVTLSKDQLSGINNIAFSN

SEQ ID NO: 6 - protein, 570 aa, Artificial Sequence
  Deletion of 137-140 (delta 4)
MELLILKANAITTILTAVTFCFASGQNITEEFYQSTCSAVSKGYLSALRTGWYTSVITIELSNIKENKCNGTDAKVKLIKQELDKYKNAVTELQLLMQSTPATNNRARRELPRFMNYTLNNAKKTNVTLSKKQKQQLLGVGSAIASGVAVSKVLHLEGEVNKIKSALLSTNKAVVSLSNGVSVLTSKVLDLKNYIDKQLLPIVNKQSCSISNIETVIEFQQKNNRLLEITREFSVNAGVTTPVSTYMLTNSELLSLINDMPITNDQKKLMSNNVQIVRQQSYSIMSIIKEEVLAYVVQLPLYGVIDTPCWKLHTSPLCTTNTKEGSNICLTRTDRGWYCDNAGSVSFFPQAETCKVQSNRVFCDTMNSLTLPSEVNLCNVDIFNPKYDCKIMTSKTDVSSSVITSLGAIVSCYGKTKCTASNKNRGIIKTFSNGCDYVSNKGVDTVSVGNTLYYVNKQEGKSLYVKGEPIINFYDPLVFPSDEFDASISQVNEKINQSLAFIRKSDELLHNVNAGKSTTNIMITTIIIVIIVILLSLIAVGLLLYCKARSTPVTLSKDQLSGINNIAFSN

SEQ ID NO: 7 - protein, 569 aa, Artificial Sequence
  Deletion of 137-141 (delta 5)
MELLILKANAITTILTAVTFCFASGQNITEEFYQSTCSAVSKGYLSALRTGWYTSVITIELSNIKENKCNGTDAKVKLIKQELDKYKNAVTELQLLMQSTPATNNRARRELPRFMNYTLNNAKKTNVTLSKKQKQQLGVGSAIASGVAVSKVLHLEGEVNKIKSALLSTNKAVVSLSNGVSVLTSKVLDLKNYIDKQLLPIVNKQSCSISNIETVIEFQQKNNRLLEITREFSVNAGVTTPVSTYMLTNSELLSLINDMPITNDQKKLMSNNVQIVRQQSYSIMSIIKEEVLAYVVQLPLYGVIDTPCWKLHTSPLCTTNTKEGSNICLTRTDRGWYCDNAGSVSFFPQAETCKVQSNRVFCDTMNSLTLPSEVNLCNVDIFNPKYDCKIMTSKTDVSSSVITSLGAIVSCYGKTKCTASNKNRGIIKTFSNGCDYVSNKGVDTVSVGNTLYYVNKQEGKSLYVKGEPIINFYDPLVFPSDEFDASISQVNEKINQSLAFIRKSDELLHNVNAGKSTTNIMITTIIIVIIVILLSLIAVGLLLYCKARSTPVTLSKDQLSGINNIAFSN

SEQ ID NO: 8 - protein, 564 aa, Artificial Sequence
  Deletion of 137-146 (delta 10)
MELLILKANAITTILTAVTFCFASGQNITEEFYQSTCSAVSKGYLSALRTGWYTSVITIELSNIKENKCNGTDAKVKLIKQELDKYKNAVTELQLLMQSTPATNNRARRELPRFMNYTLNNAKKTNVTLSKKQKQQAIASGVAVSKVLHLEGEVNKIKSALLSTNKAVVSLSNGVSVLTSKVLDLKNYIDKQLLPIVNKQSCSISNIETVIEFQQKNNRLLEITREFSVNAGVTTPVSTYMLTNSELLSLINDMPITNDQKKLMSNNVQIVRQQSYSIMSIIKEEVLAYVVQLPLYGVIDTPCWKLHTSPLCTTNTKEGSNICLTRTDRGWYCDNAGSVSFFPQAETCKVQSNRVFCDTMNSLTLPSEVNLCNVDIFNPKYDCKIMTSKTDVSSSVITSLGAIVSCYGKTKCTASNKNRGIIKTFSNGCDYVSNKGVDTVSVGNTLYYVNKQEGKSLYVKGEPIINFYDPLVFPSDEFDASISQVNEKINQSLAFIRKSDELLHNVNAGKSTTNIMITTIIIVIIVILLSLIAVGLLLYCKARSTPVTLSKDQLSGINNIAFSN

SEQ ID NO: 9 - protein, 568 aa, Artificial Sequence
  Deletion of 137-142 (delta 6)
MELLILKANAITTILTAVTFCFASGQNITEEFYQSTCSAVSKGYLSALRTGWYTSVITIELSNIKENKCNGTDAKVKLIKQELDKYKNAVTELQLLMQSTPATNNRARRELPRFMNYTLNNAKKTNVTLSKKQKQQGVGSAIASGVAVSKVLHLEGEVNKIKSALLSTNKAVVSLSNGVSVLTSKVLDLKNYIDKQLLPIVNKQSCSISNIETVIEFQQKNNRLLEITREFSVNAGVTTPVSTYMLTNSELLSLINDMPITNDQKKLMSNNVQIVRQQSYSIMSIIKEEVLAYVVQLPLYGVIDTPCWKLHTSPLCTTNTKEGSNICLTRTDRGWYCDNAGSVSFFPQAETCKVQSNRVFCDTMNSLTLPSEVNLCNVDIFNPKYDCKIMTSKTDVSSSVITSLGAIVSCYGKTKCTASNKNRGIIKTFSNGCDYVSNKGVDTVSVGNTLYYVNKQEGKSLYVKGEPIINFYDPLVFPSDEFDASISQVNEKINQSLAFIRKSDELLHNVNAGKSTTNIMITTIIIVIIVILLSLIAVGLLLYCKARSTPVTLSKDQLSGINNIAFSN

SEQ ID NO: 10 - protein, 567 aa, Artificial Sequence
  Deletion of 137-143 (delta 7)
MELLILKANAITTILTAVTFCFASGQNITEEFYQSTCSAVSKGYLSALRTGWYTSVITIELSNIKENKCNGTDAKVKLIKQELDKYKNAVTELQLLMQSTPATNNRARRELPRFMNYTLNNAKKTNVTLSKKQKQQVGSAIASGVAVSKVLHLEGEVNKIKSALLSTNKAVVSLSNGVSVLTSKVLDLKNYIDKQLLPIVNKQSCSISNIETVIEFQQKNNRLLEITREFSVNAGVTTPVSTYMLTNSELLSLINDMPITNDQKKLMSNNVQIVRQQSYSIMSIIKEEVLAYVVQLPLYGVIDTPCWKLHTSPLCTTNTKEGSNICLTRTDRGWYCDNAGSVSFFPQAETCKVQSNRVFCDTMNSLTLPSEVNLCNVDIFNPKYDCKIMTSKTDVSSSVITSLGAIVSCYGKTKCTASNKNRGIIKTFSNGCDYVSNKGVDTVSVGNTLYYVNKQEGKSLYVKGEPIINFYDPLVFPSDEFDASISQVNEKINQSLAFIRKSDELLHNVNAGKSTTNIMITTIIIVIIVILLSLIAVGLLLYCKARSTPVTLSKDQLSGINNIAFSN

SEQ ID NO: 11 - protein, 566 aa, Artificial Sequence
  Deletion of 137-144 (delta 8)
MELLILKANAITTILTAVTFCFASGQNITEEFYQSTCSAVSKGYLSALRTGWYTSVITIELSNIKENKCNGTDAKVKLIKQELDKYKNAVTELQLLMQSTPATNNRARRELPRFMNYTLNNAKKTNVTLSKKQKQQGSAIASGVAVSKVLHLEGEVNKIKSALLSTNKAVVSLSNGVSVLTSKVLDLKNYIDKQLLPIVNKQSCSISNIETVIEFQQKNNRLLEITREFSVNAGVTTPVSTYMLTNSELLSLINDMPITNDQKKLMSNNVQIVRQQSYSIMSIIKEEVLAYVVQLPLYGVIDTPCWKLHTSPLCTTNTKEGSNICLTRTDRGWYCDNAGSVSFFPQAETCKVQSNRVFCDTMNSLTLPSEVNLCNVDIFNPKYDCKIMTSKTDVSSSVITSLGAIVSCYGKTKCTASNKNRGIIKTFSNGCDYVSNKGVDTVSVGNTLYYVNKQEGKSLYVKGEPIINFYDPLVFPSDEFDASISQVNEKINQSLAFIRKSDELLHNVNAGKSTTNIMITTIIIVIIVILLSLIAVGLLLYCKARSTPVTLSKDQLSGINNIAFSN

SEQ ID NO: 12 - protein, 565 aa, Artificial Sequence
  Deletion of 137-145 (delta 9)
MELLILKANAITTILTAVTFCFASGQNITEEFYQSTCSAVSKGYLSALRTGWYTSVITIELSNIKENKCNGTDAKVKLIKQELDKYKNAVTELQLLMQSTPATNNRARRELPRFMNYTLNNAKKTNVTLSKKQKQQSAIASGVAVSKVLHLEGEVNKIKSALLSTNKAVVSLSNGVSVLTSKVLDLKNYIDKQLLPIVNKQSCSISNIETVIEFQQKNNRLLEITREFSVNAGVTTPVSTYMLTNSELLSLINDMPITNDQKKLMSNNVQIVRQQSYSIMSIIKEEVLAYVVQLPLYGVIDTPCWKLHTSPLCTTNTKEGSNICLTRTDRGWYCDNAGSVSFFPQAETCKVQSNRVFCDTMNSLTLPSEVNLCNVDIFNPKYDCKIMTSKTDVSSSVITSLGAIVSCYGKTKCTASNKNRGIIKTFSNGCDYVSNKGVDTVSVGNTLYYVNKQEGKSLYVKGEPIINFYDPLVFPSDEFDASISQVNEKINQSLAFIRKSDELLHNVNAGKSTTNIMITTIIIVIIVILLSLIAVGLLLYCKARSTPVTLSKDQLSGINNIAFSN

SEQ ID NO: 13 - protein, 565 aa, Artificial Sequence
  Deletion of 137-145 (delta 9) with wild type fusion cleavage site
MELLILKANAITTILTAVTFCFASGQNITEEFYQSTCSAVSKGYLSALRTGWYTSVITIELSNIKENKCNGTDAKVKLIKQELDKYKNAVTELQLLMQSTPATNNRARRELPRFMNYTLNNAKKTNVTLSKKRKRRSAIASGVAVSKVLHLEGEVNKIKSALLSTNKAVVSLSNGVSVLTSKVLDLKNYIDKQLLPIVNKQSCSISNIETVIEFQQKNNRLLEITREFSVNAGVTTPVSTYMLTNSELLSLINDMPITNDQKKLMSNNVQIVRQQSYSIMSIIKEEVLAYVVQLPLYGVIDTPCWKLHTSPLCTTNTKEGSNICLTRTDRGWYCDNAGSVSFFPQAETCKVQSNRVFCDTMNSLTLPSEVNLCNVDIFNPKYDCKIMTSKTDVSSSVITSLGAIVSCYGKTKCTASNKNRGIIKTFSNGCDYVSNKGVDTVSVGNTLYYVNKQEGKSLYVKGEPIINFYDPLVFPSDEFDASISQVNEKINQSLAFIRKSDELLHNVNAGKSTTNIMITTIIIVIIVILLSLIAVGLLLYCKARSTPVTLSKDQLSGINNIAFSN

SEQ ID NO: 14 - protein, 6 aa, Artificial Sequence
  mutated furin cleavage site
KKQKQQ

SEQ ID NO: 15 - protein, 6 aa, Artificial Sequence
  mutated furin cleavage site
QKQKQQ

SEQ ID NO: 16 - protein, 6 aa, Artificial Sequence
  mutated furin cleavage site
KKQKRQ

SEQ ID NO: 17 - protein, 6 aa, Artificial Sequence
  mutated furin cleavage site
GRRQQR

SEQ ID NO: 18 - protein, 6 aa, Unknown
  furin cleavage site
KKRKRR

SEQ ID NO: 19 - protein, 539 aa, Artificial Sequence
  modified RSV F protein
QNITEEFYQSTCSAVSKGYLSALRTGWYTSVITIELSNIKENKCNGTDAKVKLIKQELDKYKNAVTELQLLMQSTPATNNRARRELPRFMNYTLNNAKKTNVTLSKKQKQQAIASGVAVSKVLHLEGEVNKIKSALLSTNKAVVSLSNGVSVLTSKVLDLKNYIDKQLLPIVNKQSCSISNIETVIEFQQKNNRLLEITREFSVNAGVTTPVSTYMLTNSELLSLINDMPITNDQKKLMSNNVQIVRQQSYSIMSIIKEEVLAYVVQLPLYGVIDTPCWKLHTSPLCTTNTKEGSNICLTRTDRGWYCDNAGSVSFFPQAETCKVQSNRVFCDTMNSLTLPSEVNLCNVDIFNPKYDCKIMTSKTDVSSSVITSLGAIVSCYGKTKCTASNKNRGIIKTFSNGCDYVSNKGVDTVSVGNTLYYVNKQEGKSLYVKGEPIINFYDPLVFPSDEFDASISQVNEKINQSLAFIRKSDELLHNVNAGKSTTNIMITTIIIVIIVILLSLIAVGLLLYCKARSTPVTLSKDQLSGINNIAFSN

SEQ ID NO: 20 - protein, 25 aa, Respiratory syncytial virus
MELLILKANAITTILTAVTFCFASG